European Patent Application EP 4 711 386 A2, published March 18, 2026. Title: SITE-SPECIFIC ANTIBODY CONJUGATION AND ANTIBODY-DRUG CONJUGATE AS SPECIFIC EXAMPLE THEREOF. Applicant: AbTis co., Ltd. Application EP. The sequence listing filed with the application follows.

SEQUENCE LISTING (25 sequences)

SEQ ID NO: 1 - protein, 17 aa, synthetic construct
  REGION 1..17: note = A portion of an antibody Fc domain.
GPSVFLFPPKPKDTLMI

SEQ ID NO: 2 - protein, 9 aa, synthetic construct
  REGION 1..9: note = A motif in Fc-III.
AWHLGELVW

SEQ ID NO: 3 - protein, 9 aa, synthetic construct
  REGION 1..9: note = Synthetic sequence
  SITE 1: note = misc_feature - X can be any naturally occurring amino acid except Cysteine
  SITE 2: note = misc_feature - X can be any naturally occurring amino acid except Cysteine
  SITE 4: note = misc_feature - X is a modified amino acid Xa1 as described in Formula 3
  SITE 6: note = misc_feature - X is Glu or Asn
  SITE 9: note = misc_feature - X is Trp, Phe, or naphthylalanine
XXHXGXLVX

SEQ ID NO: 4 - protein, 9 aa, synthetic construct
  REGION 1..9: note = Synthetic sequence
  SITE 4: note = misc_feature - X is a modified amino acid Xa1 as described in Formula 3-1
  SITE 6: note = misc_feature - X is Glu or Asn
  SITE 9: note = misc_feature - X is Trp, Phe, or naphthylalanine
AWHXGXLVX

SEQ ID NO: 5 - protein, 11 aa, synthetic construct
  REGION 1..11: note = Synthetic
  SITE 1: note = misc_feature - Pro is L-proline
  SITE 2: note = misc_feature - X can be any naturally occurring amino acid except cysteine
  SITE 3: note = misc_feature - X can be any naturally occurring amino acid except cysteine
  SITE 5: note = misc_feature - X is a modified amino acid Xa1 as described in Formula 4-1
  SITE 7: note = misc_feature - X is Glu or Asn
  SITE 10: note = misc_feature - X is Trp, Phe, or naphthylalanine
  SITE 11: note = misc_feature - X is D-proline
PXXHXGXLVXP

SEQ ID NO: 6 - protein, 17 aa, synthetic construct
  REGION 1..17: note = Synthetic
  SITE 1: note = misc_feature - X can be any naturally occurring amino acid except cysteine
  SITE 2: note = misc_feature - X can be any naturally occurring amino acid except cysteine or is absent
  SITE 3: note = misc_feature - X can be any naturally occurring amino acid except cysteine or is absent
  SITE 5: note = misc_feature - X can be any naturally occurring amino acid
  SITE 6: note = misc_feature - X can be any naturally occurring amino acid
  SITE 8: note = misc_feature - X is a modified amino acid Xa1 as described in Formula 4-2
  SITE 10: note = misc_feature - X is Glu or Asn
  SITE 13: note = misc_feature - X is Trp, Phe, or naphthylalanine
  SITE 15: note = misc_feature - X can be any naturally occurring amino acid except cysteine
  SITE 16: note = misc_feature - X can be any naturally occurring amino acid except cysteine or is absent
  SITE 17: note = misc_feature - X can be any naturally occurring amino acid except cysteine or is absent
XXXCXXHXGXLVXCXXX

SEQ ID NO: 7 - protein, 15 aa, synthetic construct
  REGION 1..15: note = Synthetic
  SITE 1: note = misc_feature - Pro is L-proline
  SITE 4: note = misc_feature - X can be any naturally occurring amino acid except cysteine
  SITE 5: note = misc_feature - X can be any naturally occurring amino acid except cysteine
  SITE 7: note = misc_feature - X is a modified amino acid Xa1 as described in Formula 4-2
  SITE 9: note = misc_feature - X is Glu or Asn
  SITE 12: note = misc_feature - X is Trp, Phe, or naphthylalanine
  SITE 15: note = misc_feature - Pro is D-proline
PDCXXHXGXLVXCTP

SEQ ID NO: 8 - protein, 15 aa, synthetic construct
  REGION 1..15: note = Synthetic
  SITE 4: note = misc_feature - X can be any naturally occurring amino acid except cysteine
  SITE 5: note = misc_feature - X can be any naturally occurring amino acid except cysteine
  SITE 7: note = misc_feature - X is a modified amino acid Xa1 as described in Formula 4-2
  SITE 9: note = misc_feature - X is Glu or Asn
  SITE 12: note = misc_feature - X is Trp, Phe, or naphthylalanine
CDCXXHXGXLVXCTC

SEQ ID NO: 9 - protein, 13 aa, synthetic construct
  REGION 1..13: note = Synthetic
  SITE 3: note = misc_feature - X can be any naturally occurring amino acid except cysteine
  SITE 4: note = misc_feature - X can be any naturally occurring amino acid except cysteine
  SITE 6: note = misc_feature - X is a modified amino acid Xa1 as described in Formula 4-2
  SITE 8: note = misc_feature - X is Glu or Asn
  SITE 11: note = misc_feature - X is Trp, Phe, or naphthylalanine
DCXXHXGXLVXCT

SEQ ID NO: 10 - protein, 13 aa, synthetic construct
  REGION 1..13: note = Synthetic
  SITE 6: note = misc_feature - X is a modified amino acid Xa1 as described in Formula 4-2
DCAWHXGELVWCT

SEQ ID NO: 11 - protein, 9 aa, synthetic construct
  REGION 1..9: note = Synthetic
  SITE 1: note = misc_feature - X can be any naturally occurring amino acid except cysteine
  SITE 2: note = misc_feature - X can be any naturally occurring amino acid except cysteine
  SITE 4: note = misc_feature - X is a modified amino acid (xa1)' as described in Formula 5-1
  SITE 6: note = misc_feature - X is Glu or Asn
  SITE 9: note = misc_feature - X is Trp, Phe, or naphthylalanine
XXHXGXLVX

SEQ ID NO: 12 - protein, 17 aa, synthetic construct
  REGION 1..17: note = Synthetic
  SITE 1: note = misc_feature - X can be any naturally occurring amino acid except cysteine
  SITE 2: note = misc_feature - X can be any naturally occurring amino acid except cysteine or is absent
  SITE 3: note = misc_feature - X can be any naturally occurring amino acid except cysteine or is absent
  SITE 5: note = misc_feature - X can be any naturally occurring amino acid except cysteine
  SITE 6: note = misc_feature - X can be any naturally occurring amino acid except cysteine
  SITE 8: note = misc_feature - X is a modified amino acid (Xa1)' as described in Formula 5-2
  SITE 10: note = misc_feature - X is Glu or Asn
  SITE 13: note = misc_feature - X is Trp, Phe, or naphthylalanine
  SITE 15: note = misc_feature - X can be any naturally occurring amino acid except cysteine
  SITE 16: note = misc_feature - X can be any naturally occurring amino acid except cysteine or is absent
  SITE 17: note = misc_feature - X can be any naturally occurring amino acid except cysteine or is absent
XXXCXXHXGXLVXCXXX

SEQ ID NO: 13 - protein, 13 aa, synthetic construct
  REGION 1..13: note = Synthetic
  SITE 6: note = misc_feature - X is a modified amino acid (Xa1)' as described in Formula 5-2
DCAWHXGELVWCT

SEQ ID NO: 14 - protein, 9 aa, synthetic construct
  REGION 1..9: note = Synthetic
  SITE 1: note = misc_feature - X can be any naturally occurring amino acid except cysteine
  SITE 2: note = misc_feature - X can be one any naturally occurring amino acid except cysteine
  SITE 4: note = misc_feature - X is a modified amino acid (Xa1)' as described in Formula 6-1
  SITE 6: note = misc_feature - X is Glu or Asn
  SITE 9: note = misc_feature - X is Trp, Phe, or naphthylalanine
XXHXGXLVX

SEQ ID NO: 15 - protein, 17 aa, synthetic construct
  REGION 1..17: note = Synthetic
  SITE 1: note = misc_feature - X can be any naturally occurring amino acid except cysteine
  SITE 2: note = misc_feature - X can be any naturally occurring amino acid except cysteine or is absent
  SITE 3: note = misc_feature - X can be any naturally occurring amino acid except cysteine or is absent
  SITE 5: note = misc_feature - X can be any naturally occurring amino acid except cysteine
  SITE 6: note = misc_feature - X can be any naturally occurring amino acid except cysteine
  SITE 8: note = misc_feature - X is a modified amino acid (Xa1)' as described in Formula 6-2
  SITE 10: note = misc_feature - X is Glu or Asn
  SITE 13: note = misc_feature - X is Trp, Phe, or naphthylalanine
  SITE 15: note = misc_feature - X can be any naturally occurring amino acid except cysteine
  SITE 16: note = misc_feature - X can be any naturally occurring amino acid except cysteine or is absent
  SITE 17: note = misc_feature - X can be any naturally occurring amino acid except cysteine or is absent
XXXCXXHXGXLVXCXXX

SEQ ID NO: 16 - protein, 13 aa, synthetic construct
  REGION 1..13: note = Synthetic
  SITE 6: note = misc_feature - X is a modified amino acid (xa1)' as described in Formula 6-2
DCAWHXGELVWCT

SEQ ID NO: 17 - protein, 17 aa, synthetic construct
  REGION 1..17: note = Synthetic
  SITE 10: note = misc_feature - X is the modified amino acid (K)' as described in Formula 7-1
GPSVFLFPPXPKDTLMI

SEQ ID NO: 18 - protein, 17 aa, synthetic construct
  REGION 1..17: note = Synthetic
  SITE 12: note = misc_feature - X is the modified amino acid (K)' as described in Formula 7-2
GPSVFLFPPKPXDTLMI

SEQ ID NO: 19 - protein, 17 aa, synthetic construct
  REGION 1..17: note = Synthetic
  SITE 10: note = misc_feature - X is the modified amino acid (K)' as described in Formula 7-3
  SITE 12: note = misc_feature - X is the modified amino acid (K)' as described in Formula 7-3
GPSVFLFPPXPXDTLMI

SEQ ID NO: 20 - protein, 17 aa, synthetic construct
  REGION 1..17: note = Synthetic
  SITE 10: note = misc_feature - X is the modified amino acid (K)' as described in Formula 8-1
GPSVFLFPPXPKDTLMI

SEQ ID NO: 21 - protein, 17 aa, synthetic construct
  REGION 1..17: note = Sythetic
  SITE 12: note = misc_feature - X is the modified amino acid (K)' as described in Formula 8-2
GPSVFLFPPKPXDTLMI

SEQ ID NO: 22 - protein, 17 aa, synthetic construct
  REGION 1..17: note = Synthetic
  SITE 10: note = misc_feature - X is the modified amino acid (K)' as described in Formula 8-3
  SITE 12: note = misc_feature - X is the modified amino acid (K)' as described in Formula 8-3
GPSVFLFPPXPXDTLMI

SEQ ID NO: 23 - protein, 17 aa, synthetic construct
  REGION 1..17: note = Synthetic
  SITE 10: note = misc_feature - X is the modified amino acid (K)'' as described in Formula 10-1
GPSVFLFPPXPKDTLMI

SEQ ID NO: 24 - protein, 17 aa, synthetic construct
  REGION 1..17: note = Synthetic
  SITE 12: note = misc_feature - X is the modified amino acid (K)'' as described in Formula 10-2
GPSVFLFPPKPXDTLMI

SEQ ID NO: 25 - protein, 17 aa, synthetic construct
  REGION 1..17: note = Synthetic
  SITE 10: note = misc_feature - X is the modified amino acid (K)'' as described in Formula 10-3
  SITE 12: note = misc_feature - X is the modified amino acid (K)'' as described in Formula 10-3
GPSVFLFPPXPXDTLMI